European Patent Application EP 4 474 390 A1, published December 11, 2024. Title: HIGH AFFINITY SUMO TRAPS. Applicant: ASOCIACIÓN CENTRO DE INVESTIGACIÓN COOPERATIVA EN BIOCIENCIAS-CIC bioGUNE. The sequence listing filed with the application follows.

SEQUENCE LISTING (10 sequences)

SEQ ID NO: 1 - protein, 19 aa, synthetic construct
  source 1..19: note = small ubiquitin-related modifier (SUMO) interacting motif (SIM)
EGDEDDDIIVVDDDDDEGE

SEQ ID NO: 2 - protein, 5 aa, synthetic construct
  source 1..5: note = glycine-serine flexible linker
GGSGG

SEQ ID NO: 3 - protein, 26 aa, synthetic construct
  source 1..26: note = SIM with linkers
GSEGDEDDDIIVVDDDDDEGEGGSGG

SEQ ID NO: 4 - protein, 228 aa, synthetic construct
  source 1..228: note = GST tag
MSPILGYWKIKGLVQPTRLLLEYLEEKYEEHLYERDEGDKWRNKKFELGLEFPNLPYYIDGDVKLTQSMAIIRYIAKHNMLGGCPKERAEISMLEGAVLDIRYGVSRIAYSKDFETLKVDFLSKLPEMLKMFEDRLCHKTYLNGDHVTHPFMLYDALDVVLYMDPMCLDAFPKLVCFKKRIEAIPQIDKYLKSSKYIAWPLQGWQATFGGGDHPPKSDLEVLFGPLGS

SEQ ID NO: 5 - protein, 14 aa, Mammalian orthorubulavirus 5
GKPIPNPLLGLEST

SEQ ID NO: 6 - protein, 363 aa, synthetic construct
  source 1..363: note = SUMO-TRAP with GST and SV5
MSPILGYWKIKGLVQPTRLLLEYLEEKYEEHLYERDEGDKWRNKKFELGLEFPNLPYYIDGDVKLTQSMAIIRYIAKHNMLGGCPKERAEISMLEGAVLDIRYGVSRIAYSKDFETLKVDFLSKLPEMLKMFEDRLCHKTYLNGDHVTHPFMLYDALDVVLYMDPMCLDAFPKLVCFKKRIEAIPQIDKYLKSSKYIAWPLQGWQATFGGGDHPPKSDLEVLFGPLGSHHHHHHGSEGDEDDDIIVVDDDDDEGEGGSGGGSEGDEDDDIIVVDDDDDEGEGGSGGGSEGDEDDDIIVVDDDDDEGEGGSGGGSEGDEDDDIIVVDDDDDEGEGGSGGGSPEFPGVDLEGKPIPNPLLGLEST

SEQ ID NO: 7 - DNA, 1101 bp, synthetic construct
  source 1..1101: mol_type = other DNA; note = DNA encoding for SUMO-TRAP
atgtcccctatactaggttattggaaaattaagggccttgtgcaacccactcgacttcttttggaatatcttgaagaaaaatatgaagagcatttgtatgagcgcgatgaaggtgataaatggcgaaacaaaaagtttgaattgggtttggagtttcccaatcttccttattatattgatggtgatgttaaattaacacagtctatggccatcatacgttatatagctgacaagcacaacatgttgggtggttgtccaaaagagcgtgcagagatttcaatgcttgaaggagcggttttggatattagatacggtgtttcgagaattgcatatagtaaagactttgaaactctcaaagttgattttcttagcaagctacctgaaatgctgaaaatgttcgaagatcgtttatgtcataaaacatatttaaatggtgatcatgtaacccatcctgacttcatgttgtatgacgctcttgatgttgttttatacatggacccaatgtgcctggatgcgttcccaaaattagtttgttttaaaaaacgtattgaagctatcccacaaattgataagtacttgaaatccagcaagtatatagcatggcctttgcagggctggcaagccacgtttggtggtggcgaccatcctccaaaatcggatctggaagttctgttccaggggcccctgggatctcatcaccatcaccatcacggatctgaaggagacgaggatgacgatattatcgtagtggatgatgatgacgatgaaggagaaggtggctctggcggtggatctgaaggagacgaggatgacgatattatcgtagtggatgatgatgacgatgaaggagaaggtggctctggcggtggatctgaaggagacgaggatgacgatattatcgtagtggatgatgatgacgatgaaggagaaggtggctctggcggtggatctgaaggagacgaggatgacgatattatcgtagtggatgatgatgacgatgaaggagaaggtggctctggcggtggatccccggaattccccggggtcgacctcgagggaaagccaatacctaatccactacttggactagaatccacatag

SEQ ID NO: 8 - DNA, 78 bp, synthetic construct
  source 1..78: mol_type = other DNA; note = primer 4829
gatctgaaggagacgaggatgacgatattatcgtagtggatgatgatgacgatgaaggagaaggtggctctggcggtg

SEQ ID NO: 9 - DNA, 78 bp, synthetic construct
  source 1..78: mol_type = other DNA; note = Primer 4830
gatccaccgccagagccaccttctccttcatcgtcatcatcatccactacgataatatcgtcatcctcgtctccttca

SEQ ID NO: 10 - DNA, 18 bp, synthetic construct
  source 1..18: mol_type = other DNA; note = primer for sequencing
ggcaagccacgtttggtg